European Patent Specification EP 4 172 173 B1, published February 19, 2025. Title: NEUTROPHIL-BINDING PEPTIDES. Applicant: Yissum Research Development Company of the Hebrew Hadasit Medical Research Services and Development Ltd. The sequence listing filed with the application follows.

SEQUENCE LISTING (18 sequences)

SEQ ID NO: 1 - protein, 15 aa, Artificial
  Synthetic
KFPDLDSRRLPHMSL

SEQ ID NO: 2 - protein, 12 aa, Artificial
  Synthetic
LATTHMVFSPDH

SEQ ID NO: 3 - protein, 13 aa, Artificial
  Synthetic
PSSNLESTPLSLL

SEQ ID NO: 4 - protein, 13 aa, Artificial
  Synthetic
SSLMTTQLIATSI

SEQ ID NO: 5 - protein, 12 aa, Artificial
  Synthetic
PELDSKPYFPPL

SEQ ID NO: 6 - protein, 12 aa, Artificial
  Synthetic
ELVTASMPRPNN

SEQ ID NO: 7 - protein, 12 aa, Artificial
  Synthetic
SLESSPMAQLPQ

SEQ ID NO: 8 - protein, 12 aa, Artificial
  Synthetic
SELRSTPLLVPS

SEQ ID NO: 9 - protein, 10 aa, Artificial
  Synthetic
LQIQSWSSSP

SEQ ID NO: 10 - protein, 10 aa, Artificial
  Synthetic
STMTILGTGS

SEQ ID NO: 11 - protein, 12 aa, Artificial
  Synthetic
TETSLRIVSTNP

SEQ ID NO: 12 - protein, 12 aa, Artificial
  Synthetic
LSIVSGSALNHL

SEQ ID NO: 13 - protein, 10 aa, Artificial
  Synthetic
LTLVSERPMI

SEQ ID NO: 14 - protein, 32 aa, Artificial
  Synthetic
MLSFAAEGGQRGLQIQSWSSSPAAGADPAKAA

SEQ ID NO: 15 - protein, 19 aa, Artificial
  Synthetic
GGGSRGLQIQSWSSSPAAG

SEQ ID NO: 16 - protein, 4 aa, Artificial
  Synthetic
KAKA

SEQ ID NO: 17 - protein, 4 aa, Artificial
  Synthetic
GGGS

SEQ ID NO: 18 - protein, 5 aa, Artificial
  Synthetic
GGGGS